European Patent Specification EP 3 978 012 B1, published August 16, 2023. Title: Application of flavin-containing monooxygenase 2 (FMO2) in preparing drug for treatment of non-alcoholic fatty liver disease (NFLD). Applicant: Zhejiang University. The sequence listing filed with the application follows.

SEQUENCE LISTING (30 sequences)

SEQ ID NO: 1 - DNA, 1608 bp, Mice flavin-containing monooxygenase 2 (Mice-FMO2)
atggcaaagaaggttgtggtgattggagcaggggtcagtggcctaatctctctgaagtgctgcgtggacgagggtctggagcccacctgcttcgaaaggactgaagatatagggggactgtggagattcaaagaaaacgtggaagatggccgcgctagcatctaccgctctgtcattaccaacactagcaaagaaatgtcctgtttcagtgacttcccgatgccggaggacttccccaacttcctgcacaactctaaactcctggaatattttaggatctttgccaagaaatttgatctcctaaaatatattcagtttcagaccactgtcattagtgtgaaaaaacgcccggacttcgcatcttctgggcaatgggaagtttatactcagagcaacggaaaggagcaacgcactgtctttgacgctgttatggtttgcagcggccatcacatccagcctcacctgccactcaagtcattcccaggtattgagaggttccgaggccagtatttccatagccgcgaatacaagcacccagtggggtttgaggggaaacgcatcctggtggttggaataggaaactcagctgcagatattgcctctgaactgagtaagacggccgcgcaggtgtttgtcagcaccagacatggatcctgggtcatgagtcgaatctctgaagatggctacccttgggacatggtgttccacactagatttagctccatgctccgaaatgtcctgccccgcacggtcgtcaagtggatgatggaacaacagatgaatcgatggttcaaccatgaaaattatggtctggtgcctcagaacaaataccttatgaaagaacctgtgctaaacgacgacctccccagccgcctgctgtacggagccatcaaagtaaaaacacgggtgaaggagctcacggagacagctgtggtcttcgaggatggcacggtggaggaagacgtggatatcattgtctttgccacggggtatacgttctctttttctttcctggaagactcacttgttaaagtggaggataatagggtttccctgtacaaagccatgtttccccctcacctggagaagccaacccttgcgtgcataggtctcatccagcctctaggctccatcttcccaaccgtagagcttcaggcgcgctgggcgacaagagttttcaaaggcttgtgtagcttgccttcggagacgactatgatggcagacattgttgaaagaaatgaaaaaagagttaacctgtttgggaaaagccagagtcagatactgcagaccaactacgttgactacctggatgaactcgccttggagataggtgcaaagccagatttcgtctctctctttttcaaagaccctaaactggctgtgaaactctacttcggaccctgtaattcctaccagtaccgcctggttggacctgggcagtgggaaggagccaggaacgccatcctcacccagaagcagaggatcctgaaacccttaaagacccggactctccagtcctctgatagtgccccagtgtctttcctgctcaagatcctggggctgctcgctgttgttctggccttctttttccaacttcaggggttttaa

SEQ ID NO: 2 - protein, 535 aa, Mice flavin-containing monooxygenase 2 (Mice-FMO2)
MAKKVVVIGAGVSGLISLKCCVDEGLEPTCFERTEDIGGLWRFKENVEDGRASIYRSVITNTSKEMSCFSDFPMPEDFPNFLHNSKLLEYFRIFAKKFDLLKYIQFQTTVISVKKRPDFASSGQWEVYTQSNGKEQRTVFDAVMVCSGHHIQPHLPLKSFPGIERFRGQYFHSREYKHPVGFEGKRILVVGIGNSAADIASELSKTAAQVFVSTRHGSWVMSRISEDGYPWDMVFHTRFSSMLRNVLPRTVVKWMMEQQMNRWFNHENYGLVPQNKYLMKEPVLNDDLPSRLLYGAIKVKTRVKELTETAVVFEDGTVEEDVDIIVFATGYTFSFSFLEDSLVKVEDNRVSLYKAMFPPHLEKPTLACIGLIQPLGSIFPTVELQARWATRVFKGLCSLPSETTMMADIVERNEKRVNLFGKSQSQILQTNYVDYLDELALEIGAKPDFVSLFFKDPKLAVKLYFGPCNSYQYRLVGPGQWEGARNAILTQKQRILKPLKTRTLQSSDSAPVSFLLKILGLLAVVLAFFFQLQGF

SEQ ID NO: 3 - DNA, 1608 bp, Human flavin-containing monooxygenase 2 (Human-FMO2)
atggcaaagaaggtagctgtgattggagctggggtcagtggcctaatttctctgaagtgctgtgtggatgagggacttgagcccacttgctttgagagaactgaagatattggaggagtgtggaggttcaaagagaatgtggaagatggccgagcaagtatctatcaatctgtcgttaccaacaccagcaaagaaatgtcctgtttcagtgactttccaatgcctgaagattttccaaacttcctgcataattctaaacttctggaatatttcaggatttttgctaaaaaatttgatctgctaaaatatattcagttccagacaactgtccttagtgtgagaaaatgtccagatttctcatcctctggccaatggaaggttgtcactcagagcaacggcaaggagcagagtgctgtctttgacgcagttatggtttgcagtggccaccacattctacctcatatcccactgaagtcatttccaggtatggagaggttcaaaggccaatatttccatagccgccaatacaagcatccagatggatttgagggaaaacgcatcctggtgattggaatgggaaactcaggctcagatattgctgttgagctgagtaagaatgctgctcaggtttttatcagcaccaggcatggcacctgggtcatgagccgtatctctgaagatggctatccttgggactcagtgttccacacccggtttcgttctatgctccgcaatgtactgccacgaacagctgtaaaatggatgatagaacaacagatgaatcggtggttcaaccatgaaaattatggccttgagcctcaaaacaaatacattatgaaggaacctgtactaaatgatgatgtcccaagtcgtctactctgtggagccatcaaggtgaaatctacagtgaaagagctcacagaaacttctgccatctttgaggatggaacagtggaggagaacattgatgtcatcatttttgcaacaggatatagtttctcttttcccttccttgaagattcactcgttaaagtagagaataatatggtctcactgtataaatacatattccccgctcacctggacaagtcaaccctcgcgtgcattggtctcatccagcccctaggttccattttcccaactgctgaacttcaagctcgttgggtgacaagagttttcaaaggcttgtgtagcctgccctcagagagaactatgatgatggacattatcaaaaggaatgaaaaaagaattgacctgtttggagaaagccagagccagacgttgcagaccaattatgttgactacttggacgagctcgccttagagataggtgcgaagccagatttctgctctctcttgttcaaagatcctaaactggctgtgagactctatttcggaccctgcaactcctatcagtatcgcctggttgggcctgggcaatgggaaggagccagaaatgccatcttcacccagaaacaaagaatactgaagccactcaagactcgggccctgaaggattcatctaatttctcagtttcttttctgttgaaaatcctgggccttcttgctgttgttgtggcctttttttgccaacttcaatggtcctag

SEQ ID NO: 4 - protein, 535 aa, Human flavin-containing monooxygenase 2 (Human-FMO2) [sequence omitted]

SEQ ID NO: 5 - DNA, 20 bp, ACTIN-F(primer sequence ACTIN-F)
acactgtgcccatctacgag

SEQ ID NO: 6 - DNA, 21 bp, ACTIN-R(primer sequence ACTIN-R)
cagcactgtgttggcatagag

SEQ ID NO: 7 - DNA, 23 bp, HMGCR-F(primer sequence HMGCR-F)
atcatgtgctgcttcggctgcat

SEQ ID NO: 8 - DNA, 22 bp, HMGCR-R(primer sequence HMGCR-R)
aaattggacgaccctcacggct

SEQ ID NO: 9 - DNA, 22 bp, CYP7A1-F(primer sequence CYP7A1-F)
tcaaagagcgctgtctgggtca

SEQ ID NO: 10 - DNA, 22 bp, CYP7A1-R(primer sequence CYP7A1-R)
tttcccgggctttatgtgcggt

SEQ ID NO: 11 - DNA, 22 bp, ABCG1-F(primer sequence ABCG1-F)
tgaacccgtttctttggcaccg

SEQ ID NO: 12 - DNA, 22 bp, ABCG1-R(primer sequence ABCG1-R)
agtcccgcatgatgctgaggaa

SEQ ID NO: 13 - DNA, 22 bp, FATP1-F(primer sequence FATP1-F)
tgcacagcaggtactaccgcat

SEQ ID NO: 14 - DNA, 20 bp, FATP1-R(primer sequence FATP1-R)
tgcgcagtaccaccgtcaac

SEQ ID NO: 15 - DNA, 22 bp, FABP1-F(primer sequence FABP1-F)
tggtccgcaatgagttcaccct

SEQ ID NO: 16 - DNA, 24 bp, FABP1-R(primer sequence FABP1-R)
ccagcttgacgactgccttgactt

SEQ ID NO: 17 - DNA, 20 bp, SREBP1c-F(primer sequence SREBP1c-F)
ggagccatggattgcacatt

SEQ ID NO: 18 - DNA, 20 bp, SREBP1c-R(primer sequence SREBP1c-R)
gcttccagagaggaggccag

SEQ ID NO: 19 - DNA, 24 bp, FASN-F(primer sequence FASN-F)
tccaagactgactcggctactgac

SEQ ID NO: 20 - DNA, 23 bp, FASN-R(primer sequence FASN-R)
gcagccaggttcggaatgctatc

SEQ ID NO: 21 - DNA, 20 bp, PDK4-F(primer sequence PDK4-F)
ttcacaccttcaccacatgc

SEQ ID NO: 22 - DNA, 20 bp, PDK4-R(primer sequence PDK4-R)
aaagggcggttttcttgatg

SEQ ID NO: 23 - DNA, 16 bp, CPT1-F(primer sequence CPT1-F)
accactggccgcatgt

SEQ ID NO: 24 - DNA, 21 bp, CPT1-R(primer sequence CPT1-R)
ctccatggcgtagtagttgct

SEQ ID NO: 25 - DNA, 22 bp, ACOX1-F(primer sequence ACOX1-F)
cggaagatacataaaggagacc

SEQ ID NO: 26 - DNA, 21 bp, ACOX1-R(primer sequence ACOX1-R)
aagtaggacaccataccaccc

SEQ ID NO: 27 - DNA, 20 bp, MCAD-F(primer sequence MCAD-F)
gctagtggagcaccaaggag

SEQ ID NO: 28 - DNA, 20 bp, MCAD-R(primer sequence MCAD-R)
ccaggctgctctctggtaac

SEQ ID NO: 29 - DNA, 20 bp, UCP2-F(primer sequence UCP2-F)
gctggtggtggtcggagata

SEQ ID NO: 30 - DNA, 19 bp, UCP2-R(primer sequence UCP2-R)
actggcccaaggcagagtt